European Patent Application EP 4 201 924 A1, published June 28, 2023. Title: IRE1 SMALL MOLECULE INHIBITORS. Applicant: Cornell University. Application EP. The sequence listing filed with the application follows.

SEQUENCE LISTING (28 sequences)

SEQ ID NO: 1 - protein, 977 aa, Homo sapiens
MPARRLLLLLTLLLPGLGIFGSTSTVTLPETLLFVSTLDGSLHAVSKRTGSIKWTLKEDPVLQVPTHVEEPAFLPDPNDGSLYTLGSKNNEGLTKLPFTIPELVQASPCRSSDGILYMGKKQDIWYVIDLLTGEKQQTLSSAFADSLCPSTSLLYLGRTEYTITMYDTKTRELRWNATYFDYAASLPEDDVDYKMSHFVSNGDGLVVTVDSESGDVLWIQNYASPVVAFYVWQREGLRKVMHINVAVETLRYLTFMSGEVGRITKWKYPFPKETEAKSKLTPTLYVGKYSTSLYASPSMVHEGVAVVPRGSTLPLLEGPQTDGVTIGDKGECVITPSTDVKFDPGLKSKNKLNYLRNYWLLIGHHETPLSASTKMLERFPNNLPKHRENVIPADSEKKSFEEVINLVDQTSENAPTTVSRDVEEKPAHAPARPEAPVDSMLKDMATIILSTFLLIGWVAFIITYPLSMHQQQQLQHQQFQKELEKIQLLQQQQQQLPFHPPGDTAQDGELLDTSGPYSESSGTSSPSTSPRASNHSLCSGSSASKAGSSPSLEQDDGDEETSVVIVGKISFCPKDVLGHGAEGTIVYRGMFDNRDVAVKRILPECFSFADREVQLLRESDEHPNVIRYFCTEKDRQFQYIAIELCAATLQEYVEQKDFAHLGLEPITLLQQTTSGLAHLHSLNIVHRDLKPHNILISMPNAHGKIKAMISDFGLCKKLAVGRHSFSRRSGVPGTEGWIAPEMLSEDCKENPTYTVDIFSAGCVFYYVISEGSHPFGKSLQRQANILLGACSLDCLHPEKHEDVIARELIEKMIAMDPQKRPSAKHVLKHPFFWSLEKQLQFFQDVSDRIEKESLDGPIVKQLERGGRAVVKMDWRENITVPLQTDLRKFRTYKGGSVRDLLRAMRNKKHHYRELPAEVRETLGSLPDDFVCYFTSRFPHLLAHTYRAMELCSHERLFQPYYFHEPPEPQPPVTPDAL

SEQ ID NO: 2 - RNA, 17 nt, synthetic construct
  source 1..17: mol_type = other RNA
catgtccgcagcacatg

SEQ ID NO: 3 - RNA, 17 nt, synthetic construct
  source 1..17: mol_type = other RNA
catgtccccagcacatg

SEQ ID NO: 4 - protein, 434 aa, Saccharomyces cerevisiae
SRIANIPNFEQSLKNLVVSEKILGYGSSGTVVFQGSFQGRPVAVKRMLIDFCDIALMEIKLLTESDDHPNVIRYYCSETTDRFLYIALELCNLNLQDLVESKNVSDENLKLQKEYNPISLLRQIASGVAHLHSLKIIHRDLKPQNILVSTSSRFTADQQTGAENLRILISDFGLCKKLDSGQSSFRTNLNNPSGTSGWRAPELLEESNNLQTKRRLTRSIDIFSMGCVFYYILSKGKHPFGDKYSRESNIIRGIFSLDEMKCLHDRSLIAEATDLISQMIDHDPLKRPTAMKVLRHPLFWPKSKKLEFLLKVSDRLEIENRDPPSALLMKFDAGSDFVIPSGDWTVKFDKIFMDNLERYRKYHSSKLMDLLRALRNKYHHFMDLPEDIAELMGPVPDGFYDYFIKRFPNLLIGVYMIVKENLSDDQILREFLYS

SEQ ID NO: 5 - protein, 424 aa, Homo sapiens
DDGDEETSVVIVGKISFCPKDVLGHGAEGTIVYRGMFDNRDVAVKRILPECFSFADREVQLLRESDEHPNVIRYFCTEKDRQFQYIAIELCAATLQEYVEQKDCFAHLGLEPITLLQQTTSGLAHLHSLNIVHRDLKPHNILISMPNAHGKIKAMISDFGLCKKLAVGRHSFSRRSGVPGTEGWIAPEMLSEDCKENPTYTVDIFSAGCVFYYVVSEGSHPFGKSLQRQANILLGACSLDCLHPEKHEDVIARELIEKMIAMDPQKRPSANDVLKHPFFWSLEKQLQFFQDVSDRIEKESLDGPIVKQLERGGRAVVKMDWRENITDPLQTDLRKFRTYKGGSVRDLLRAMRNKKHHYRDLPEEVRETLGTLPDDFVCYFTSRFPHLLAHTYRAMELCSHERLFQPYYFHEPPEPQPPVTPDAL

SEQ ID NO: 6 - protein, 423 aa, Mus musculus
DDEDEETRMVIVGKISFCPKDVLGHGAEGTIVYKGMFDNRDVAVKRILPECFSFADREVQLLRESDEHPNVIRYFCTEKDRQFQYIAIELCAATLQEYVEQKDFAHLGLEPITLLHQTTSGLAHLHSLNIVHRDLKPHNILLSMPNAHGRIKAMISDFGLCKKLAVGRHSFSRRSGVPGTEGWIAPEMLSEDCKDNPTYTVDIFSAGCVFYYVISEGNHPFGKSLQRQANILLGACNLDCFHSDKHEDVIARELIEKMIAMDPQQRPSAKHVLKHPFFWSLEKQLQFFQDVSDRIEKEALDGPIVRQLERGGRAVVKMDWRENITVPLQTDLRKFRTYKGGSVRDLLRAMRNKKHHYRELPAEVQETLGSIPDDFVRYFTSRFPHLLSHTYQAMELCRHERLFQTYYWHEPTEPQPPVIPYAL

SEQ ID NO: 7 - protein, 423 aa, Rattus norvegicus
DDEDEETRMVIVGKISFCPKDVLGHGAEGTIVYKGMFDNRDVAVKRILPECFSFADREVQLLRESDEHPNVIRYFCTEKDRQFQYIAIELCAATLQEYVEQKDFAHLGLEPITLLHQTTSGLAHLHSLNIVHRDLKPHNILLSMPNAHGRIKAMISDFGLCKKLAVGRHSFSRRSGVPGTEGWIAPEMLSEDCKENPTYTVDIFSAGCVFYYVISEGNHPFGKSLQRQANILLGACSLDCFHSDKHEDVIARELIEKMIAMDPQQRPSAKHVLKHPFFWSLEKQLQFFQDVSDRIEKESLDGPIVRQLERGGRAVVKMDWRENITVPLQTDLRKFRTYKGGSVRDLLRAMRNKRHHYRELPLEVQETLGSIPDDFVRYFTSRFPHLLSHTYRAMELCRHERLFQTYYWHEPTEAQPPGIPDAL

SEQ ID NO: 8 - DNA, 20 bp, synthetic construct
  source 1..20: mol_type = other DNA
acacgtttgggaatggacac

SEQ ID NO: 9 - DNA, 20 bp, synthetic construct
  source 1..20: mol_type = other DNA
ccatgggaagatgttctggg

SEQ ID NO: 10 - DNA, 24 bp, synthetic construct
  source 1..24: mol_type = other DNA
ctcaggaggagcaatgatcttgat

SEQ ID NO: 11 - DNA, 20 bp, synthetic construct
  source 1..20: mol_type = other DNA
taccaccatgtacccaggca

SEQ ID NO: 12 - DNA, 23 bp, synthetic construct
  source 1..23: mol_type = other DNA
gacagagagtcaaactaacgtgg

SEQ ID NO: 13 - DNA, 19 bp, synthetic construct
  source 1..19: mol_type = other DNA
gtccagcaggcaagaaggt

SEQ ID NO: 14 - DNA, 20 bp, synthetic construct
  source 1..20: mol_type = other DNA
aagaacacgcttgggaatgg

SEQ ID NO: 15 - DNA, 17 bp, synthetic construct
  source 1..17: mol_type = other DNA
ctgcacctgctgcggac

SEQ ID NO: 16 - DNA, 18 bp, synthetic construct
  source 1..18: mol_type = other DNA
cctgagcccggaggagaa

SEQ ID NO: 17 - DNA, 18 bp, synthetic construct
  source 1..18: mol_type = other DNA
ctcgagcagtctgcgctg

SEQ ID NO: 18 - DNA, 21 bp, synthetic construct
  source 1..21: mol_type = other DNA
taaaagccctgatgctgaagc

SEQ ID NO: 19 - DNA, 19 bp, synthetic construct
  source 1..19: mol_type = other DNA
tccgactattggcatccga

SEQ ID NO: 20 - DNA, 21 bp, synthetic construct
  source 1..21: mol_type = other DNA
ctatttccagggcttccgagt

SEQ ID NO: 21 - DNA, 21 bp, synthetic construct
  source 1..21: mol_type = other DNA
aggtgttgtactggcctcggt

SEQ ID NO: 22 - DNA, 19 bp, synthetic construct
  source 1..19: mol_type = other DNA
aagccctctggaacttgcg

SEQ ID NO: 23 - DNA, 19 bp, synthetic construct
  source 1..19: mol_type = other DNA
aacccaatggcctgtctgg

SEQ ID NO: 24 - DNA, 19 bp, synthetic construct
  source 1..19: mol_type = other DNA
tcatcggacgcacttggaa

SEQ ID NO: 25 - DNA, 21 bp, synthetic construct
  source 1..21: mol_type = other DNA
caaccaccttgaatggcaaga

SEQ ID NO: 26 - DNA, 21 bp, synthetic construct
  source 1..21: mol_type = other DNA
gtccctagcttggctgacaga

SEQ ID NO: 27 - DNA, 18 bp, synthetic construct
  source 1..18: mol_type = other DNA
tggagagcgagggctttg

SEQ ID NO: 28 - DNA, 21 bp, synthetic construct
  source 1..21: mol_type = other DNA
agcttgattgtcaacctcctg